European Patent Application EP 4 779 031 A2, published July 22, 2026. Title: COMPOSITIONS AND METHODS FOR MAKING CONTROLS FOR SEQUENCE-BASED GENETIC TESTING. Applicant: Illumina, Inc. Application EP. The sequence listing filed with the application follows.

SEQUENCE LISTING (6 sequences)

SEQ ID NO: 1 - DNA, 42 bp, synthetic construct
  misc_feature 1..42: note = source = /note="Description of Artificial Sequence: Synthetic primer"
  source 1..42: mol_type = other DNA
aatgatacggcgaccaccgacttgaggtcggatagctcttct

SEQ ID NO: 2 - DNA, 45 bp, synthetic construct
  source 1..45: mol_type = other DNA
  misc_feature 1..45: note = source = /note="Description of Artificial Sequence: Synthetic primer"
  modified_base 1: mod_base = OTHER; note = 5' Phosphorylation (/5Phos/)
gaagagctatccgacctcaagatctcgtatgccgtcttctgcttg

SEQ ID NO: 3 - DNA, 170 bp, synthetic construct
  misc_feature 1..170: note = source = /note="Description of Artificial Sequence: Synthetic primer"
  source 1..170: mol_type = other DNA
gtcggatagcgccactatgagcatattcggtttacctcagattgtataattgatgacgataaacattcaccggagaagatctaacgtaagtatatagttataactgaaccgttcgaacacttactccgtttacttaattacgccttactgtcatgcctggctcgtaagtt

SEQ ID NO: 4 - DNA, 170 bp, synthetic construct
  misc_feature 1..170: note = source = /note="Description of Artificial Sequence: Synthetic primer"
  source 1..170: mol_type = other DNA
aacttacgagccaggcatgacagtaaggcgtaattaagtaaacggagtaagtgttcgaacggttcagttataactatatacttacgttagatcttctccggtgaatgtttatcgtcatcaattatacaatctgaggtaaaccgaatatgctcatagtggcgctatccgac

SEQ ID NO: 5 - DNA, 26 bp, synthetic construct
  misc_feature 1..26: note = source = /note="Description of Artificial Sequence: Synthetic primer"
  source 1..26: mol_type = other DNA
  modified_base 1: mod_base = OTHER; note = 5' Inverted Dideoxy-T (/5InvddT/)
taacttacgagccaggcatgacagta

SEQ ID NO: 6 - DNA, 26 bp, synthetic construct
  misc_feature 1..26: note = source = /note="Description of Artificial Sequence: Synthetic primer"
  source 1..26: mol_type = other DNA
  modified_base 1: mod_base = OTHER; note = 5' Inverted Dideoxy-T (/5InvddT/)
tgtcggatagcgccactatgagcata